European Patent Application EP 4 450 614 A1, published October 23, 2024. Title: Treatment of leukemia by combining a hypomethylating agent in combination with engineered CAR-NK cells. Applicant: Johann Wolfgang Goethe-Universität Frankfurt am Main. Application EP. The sequence listing filed with the application follows.

SEQUENCE LISTING (4 sequences)

SEQ ID NO: 1 - protein, 265 aa, Homo sapiens
MSEEVTYADLQFQNSSEMEKIPEIGKFGEKAPPAPSHVWRPAALFLTLLCLLLLIGLGVLASMFHVTLKIEMKKMNKLQNISEELQRNISLQLMSNMNISNKIRNLSTTLQTIATKLCRELYSKEQEHKCKPCPRRWIWHKDSCYFLSDDVQTWQESKMACAAQNASLLKINNKNALEFIKSQSRSYDYWLGLSPEEDSTRGMRVDNIINSSAWVIRNAPDLNNMYCGYINRLYVQYYHCTYKKRMICEKMANPVQLGSTYFREA

SEQ ID NO: 2 - protein, 493 aa, synthetic construct
DIQMTQSPSSLSASVGDRVTITCRASQSISSYLNWYQQKPGKAPKLLIYAASSLQSGVPSRFSGSGSGTDFTLTISSLQPEDFATYYCQQSYSTPPTFGQGTKVEIKGGGGSGGGGSGGGGSQVQLVQSGAEVKKPGASVKVSCKASGYTFTSYYMHWVRQAPGQGLEWMGIINPSGGSTSYAQKFQGRVTMTRDTSTSTVYMELSSLRSEDTAVYYCAKGTTGDWFDYWGQGTLVTVSSEQKLISEEDLALSNSIMYFSHFVPVFLPAKPTTTPAPRPPTPAPTIASQPLSLRPEASRPAAGGAVHTRGLDFACDIYIWAPLAGTCGVLLLSLVITLYKRGRKKLLYIFKQPFMRPVQTTQEEDGCSCRFPEEEEGGCELRVKFSRSADAPAYQQGQNQLYNELNLGRREEYDVLDKRRGRDPEMGGKPRRKNPQEGLYNELQKDKMAEAYSEIGMKGERRRGKGHDGLYQGLSTATKDTYDALHMQALPPR

SEQ ID NO: 3 - protein, 443 aa, synthetic construct
DIQMTQSPSSLSASVGDRVTITCRASQSISSYLNWYQQKPGKAPKLLIYAASSLQSGVPSRFSGSGSGTDFTLTISSLQPEDFATYYCQQSYSTPPTFGQGTKVEIKGGGGSGGGGSGGGGSQVQLVQSGAEVKKPGASVKVSCKASGYTFTSYYMHWVRQAPGQGLEWMGIINPSGGSTSYAQKFQGRVTMTRDTSTSTVYMELSSLRSEDTAVYYCAKGTTGDWFDYWGQGTLVTVSSEQKLISEEDLESKYGPPCPSCPFACDIYIWAPLAGTCGVLLLSLVITLYKRGRKKLLYIFKQPFMRPVQTTQEEDGCSCRFPEEEEGGCELRVKFSRSADAPAYQQGQNQLYNELNLGRREEYDVLDKRRGRDPEMGGKPRRKNPQEGLYNELQKDKMAEAYSEIGMKGERRRGKGHDGLYQGLSTATKDTYDALHMQALPPR

SEQ ID NO: 4 - protein, 27 aa, synthetic construct
FACDIYIWAPLAGTCGVLLLSLVITLY